European Patent Specification EP 3 336 099 B1, published March 4, 2026. Title: Verfahren zur selektiven Immobilisierung von Zellen auf einem festen Tägermaterial und diese umfassende Vorrichtungen. Applicant: Karlsruher Institut für Technologie. The sequence listing filed with the application follows.

SEQUENCE LISTING (40 sequences)

SEQ ID NO: 1 - protein, 5 aa, Artificial sequence
  Peptidlinker
GGGGS

SEQ ID NO: 2 - DNA, 94 bp, Artificial sequence
  PCR-Primer (TP1)
ttccagttcaccagccagaccttcaacaacgtgaccaccacgccaaccggtggttttttcgtccatgctaccaccaccacccacaccattatcc

SEQ ID NO: 3 - DNA, 95 bp, Artificial sequence
  PCR-Primer (TP2)
ctggtgaactggaacagctgcgtgctcgtctggaacaccacccgcagggtcagcgtgaaccctaatgagatccggctgctaacaaagcccgaaag

SEQ ID NO: 4 - DNA, 30 bp, Artificial sequence
  PCR-Primer (TP3)
tgagatccggctgctaacaaagcccgaaag

SEQ ID NO: 5 - DNA, 28 bp, Artificial sequence
  PCR-Primer (TP4)
gctaccaccaccacccacaccattatcc

SEQ ID NO: 6 - DNA, 53 bp, Artificial sequence
  PCR-Primer (TP5)
ccggataatggtgtgggtggtggtggtagcgttgataccctgagcggtctgag

SEQ ID NO: 7 - DNA, 59 bp, Artificial sequence
  PCR-Primer (TP6)
tcgggctttgttagcagccggatctcattaaatatgtgcatcacctttggttgctttac

SEQ ID NO: 8 - DNA, 62 bp, Artificial sequence
  PCR-Primer (TP7)
tataggcatcaaccataacaatatgtgcatgtatatctccttcttaaagttaaacaaaatta

SEQ ID NO: 9 - DNA, 49 bp, Artificial sequence
  PCR-Primer (TP8)
ttatggttgatgcctataaaccgaccaaaggtggtggtggcagcgttag

SEQ ID NO: 10 - DNA, 61 bp, Artificial sequence
  PCR-Primer (TP11)
ggatgattctggtaacagggaatgtgattgaattttgtttaactttaagaaggagatatac

SEQ ID NO: 11 - DNA, 50 bp, Artificial sequence
  PCR-Primer (TP12)
ctaacaccgaaagaggcttttcgcacggttgcaaaaaacccctcaagacc

SEQ ID NO: 12 - DNA, 18 bp, Artificial sequence
  PCR-Primer (TP13)
aaccgtgcgaaaagcctc

SEQ ID NO: 13 - DNA, 22 bp, Artificial sequence
  PCR-Primer (TP14)
caatcacattccctgttaccag

SEQ ID NO: 14 - DNA, 20 bp, Artificial sequence
  PCR-Primer (41_KSR23_for)
gatccggctgctaacaaagc

SEQ ID NO: 15 - DNA, 31 bp, Artificial sequence
  PCR-Primer (42_KSR23_rev)
gttaaacaaaattatttctagaggggaattg

SEQ ID NO: 16 - DNA, 23 bp, Artificial sequence
  PCR-Primer (124_KSR65_for)
gatccggctgctaacaaagcccg

SEQ ID NO: 17 - DNA, 46 bp, Artificial sequence
  PCR-Primer (125_KSR65_rev)
atgtatatctccttcttaaagttaaacaaaattatttctagagggg

SEQ ID NO: 18 - DNA, 27 bp, Artificial sequence
  PCR-Primer (380_KSR205-for)
taatgagatccggctgctaacaaagcc

SEQ ID NO: 19 - DNA, 23 bp, Artificial sequence
  PCR-Primer (381_KSR205-rev)
gctaccaccaccacccacaccat

SEQ ID NO: 20 - DNA, 56 bp, Artificial sequence
  PCR-Primer (382_KSR206-for)
cacccgtccggataatggtgtgggtggtggtggtagcgaaattggcaccggttttc

SEQ ID NO: 21 - DNA, 56 bp, Artificial sequence
  PCR-Primer (383_KSR206-rev)
ctttcgggctttgttagcagccggatctcattaaccgccgctaatttccagggtgc

SEQ ID NO: 22 - DNA, 29 bp, Artificial sequence
  PCR Primer (KSR_168)
cgtgattttgcaggagacgggttagttac

SEQ ID NO: 23 - DNA, 36 bp, Artificial sequence
  PCR Primer (KSR_169)
gtctcctgcaaaatcacgtacaaatttaagaccttg

SEQ ID NO: 24 - DNA, 71 bp, Artificial sequence
  PCR Primer (MS1)
ggggacaagtttgtacaaaaaagcaggctctgaaaacctgtattttcagtgctcagtttttgtttcaggtg

SEQ ID NO: 25 - DNA, 56 bp, Artificial sequence
  PCR Primer (MS2)
ggggaccactttgtacaagaaagctgggtgttatattctgccctcaaattttaaaa

SEQ ID NO: 26 - DNA, 27 bp, Artificial sequence
  PCR Primer (TP17)
gctaccaccaccacccacaccattatc

SEQ ID NO: 27 - DNA, 26 bp, Artificial sequence
  PCR Primer (TP18)
taatgagatccggctgctaacaaagc

SEQ ID NO: 28 - DNA, 55 bp, Artificial sequence
  PCR Primer (TP19)
ccggataatggtgtgggtggtggtggtagctcagtttttgtttcaggtgctaacg

SEQ ID NO: 29 - DNA, 54 bp, Artificial sequence
  PCR Primer (TP20)
tcgggctttgttagcagccggatctcattatattctgccctcaaattttaaaat

SEQ ID NO: 30 - DNA, 57 bp, Artificial sequence
  PCR Primer (TP25)
atgatggtggtgatgatgcatgtatatctccttcttaaagttaaacaaaattatttc

SEQ ID NO: 31 - DNA, 51 bp, Artificial sequence
  PCR Primer (TP26)
catcatcaccaccatcatgcacatattgttatggttgatgcctataaaccg

SEQ ID NO: 32 - DNA, 50 bp, Artificial sequence
  PCR Primer (TP27)
ctttaagaaggaatatcacaagtttgtactaagaaggagatatacatatg

SEQ ID NO: 33 - DNA, 46 bp, Artificial sequence
  PCR Primer (TP28)
ggtggtggtggtagcgcccatattgttatggtggatgcatataaac

SEQ ID NO: 34 - DNA, 59 bp, Artificial sequence
  PCR-Primer (TP35)
agtttgtactaagaaggagatatacatatgacaattaaagaaatgcctcagccaaaaac

SEQ ID NO: 35 - DNA, 51 bp, Artificial sequence
  PCR Primer (TP36)
cataacaatatgggcgctaccaccaccacccccagcccacacgtcttttgc

SEQ ID NO: 36 - DNA, 50 bp, Artificial sequence
  PCR Primer (SG3)
gggcatcatcaccaccatcattaatgagatccggctgctaacaaagcccg

SEQ ID NO: 37 - DNA, 42 bp, Artificial sequence
  PCR Primer (SG4)
ttaatgatggtggtgatgatgcccagcccacacgtcttttgc

SEQ ID NO: 38 - DNA, 59 bp, Artificial sequence
  PCR Primer (SG7)
tataaaccgaccaaaggtggtggtggcagcacaattaaagaaatgcctcagccaaaaac

SEQ ID NO: 39 - DNA, 51 bp, Artificial sequence
  PCR Primer (SG8)
ctttcgggctttgttagcagccggatcttacccagcccacacgtcttttgc

SEQ ID NO: 40 - DNA, 22 bp, Artificial sequence
  kommerziell erhältliches Oligonukleotid Cy5-F5-AmC7
ggtccggtcataaagcgataag